European Patent Application EP 4 473 973 A1, published December 11, 2024. Title: VIPR2 antagonist peptide for inhibiting cancer metastasis. Applicant: 一丸ファルコス株式会社. The sequence listing filed with the application follows.

SEQUENCE LISTING (3 sequences)

SEQ ID NO: 1 - protein, 13 aa, synthetic construct
  MOD_RES 1: note = 3-mercaptopropanoic acid (Mpa)
  DISULFID 1..10: note = disulfide bond
  CROSSLNK 7..11: note = Cyclization by amide linkage
  MOD_RES 13: note = AMIDATION
XPPYLPKYLCDLI

SEQ ID NO: 2 - protein, 13 aa, synthetic construct
  MOD_RES 1: note = ACETYLATION
  DISULFID 1..10: note = disulfide bond
  CROSSLNK 7..11: note = Cyclization by amide linkage
  MOD_RES 13: note = AMIDATION
CPPYLPKYLCDLI

SEQ ID NO: 3 - protein, 13 aa, synthetic construct
  VARIANT 1: note = C,3-mercaptopropionic acid(Mpa),D-cysteine; note = N-terminus amino group is optionally modified or deleted
  VARIANT 3: note = MeGly,N-methylated alanine,2-azetidine-2-carboxylic acid,P,Hydroxyproline,3,4-dehydroproline,Pipecolic acid,S,K
  VARIANT 8: note = Y,P,R
  VARIANT 7: note = K,Orn,D,E; note = X7 and X11 represent any combination of lysine and aspartic acid, ornithine and glutamic acid, aspartic acid and lysine, glutamic acid and ornithine, lysine and glutamic acid, or glutamic acid and lysine
  VARIANT 11: note = D,E,K,Orn; note = X7 and X11 represent any combination of lysine and aspartic acid, ornithine and glutamic acid, aspartic acid and lysine, glutamic acid and ornithine, lysine and glutamic acid, or glutamic acid and lysine
  VARIANT 12: note = L,I,Nle
  VARIANT 13: note = L,I,Nle; note = C-terminus carboxy group is optionally modified or deleted
  DISULFID 1..10: note = disulfide bond
  CROSSLNK 7..11: note = Cyclization by amide linkage
XPXYLPXXLCXXX